European Patent Application EP 4 644 545 A1, published November 5, 2025. Title: Method for preparing circular RNA using dumbbell structure. Applicant: RiboTech Inc. Application KR. The sequence listing filed with the application follows.

SEQUENCE LISTING (45 sequences)

SEQ ID NO: 1 - DNA, 58 bp, synthetic construct
  misc_feature 1..58: note = pUC-DB primer_F for preparing pUC-3'DB
  source 1..58: mol_type = other DNA
gcgctgtttaaactaatacgactcactataggaaaaaatcgagggtctcccctagttg

SEQ ID NO: 2 - DNA, 31 bp, synthetic construct
  misc_feature 1..31: note = pUC-DB primer_R for preparing pUC-3'DB
  source 1..31: mol_type = other DNA
gcgctgcgatcgcccattttgctgtattcaa

SEQ ID NO: 3 - DNA, 82 bp, synthetic construct
  misc_feature 1..82: note = pUC-3'DB primer_F for preparing 3'DB-M1
  source 1..82: mol_type = other DNA
ctttgtttaaactaatacgactcactataggaaaaatccctagttgttgtgtggacaaaacacagcggccgcttaaaacagc

SEQ ID NO: 4 - DNA, 51 bp, synthetic construct
  misc_feature 1..51: note = pUC-3'DB primer_R for preparing 3'DB-M1
  source 1..51: mol_type = other DNA
tggactagttgttgtgtgggtcgacttttgttttttgttttttttttgttt

SEQ ID NO: 5 - DNA, 77 bp, synthetic construct
  misc_feature 1..77: note = pUC-3'DB primer_F for preparing 3'DB-M2
  source 1..77: mol_type = other DNA
ctttgtttaaactaatacgactcactataggaaaaatccctagttgtggacaaaacacagcggccgcttaaaacagc

SEQ ID NO: 6 - DNA, 45 bp, synthetic construct
  misc_feature 1..45: note = pUC-3'DB primer_R for preparing 3'DB-M2
  source 1..45: mol_type = other DNA
tggactagttgtgggtcgacttttgttttttgttttttttttgtt

SEQ ID NO: 7 - DNA, 77 bp, synthetic construct
  misc_feature 1..77: note = pUC-3'DB primer_F for preparing 3'DB-M3
  source 1..77: mol_type = other DNA
ctttgtttaaactaatacgactcactataggaaaaatccctagtcgcggacaaaacacagcggccgcttaaaacagc

SEQ ID NO: 8 - DNA, 46 bp, synthetic construct
  misc_feature 1..46: note = pUC-3'DB primer_R for preparing 3'DB-M3
  source 1..46: mol_type = other DNA
tggactagtcgcgggtcgacttttgttttttgttttttttttgttt

SEQ ID NO: 9 - DNA, 56 bp, synthetic construct
  misc_feature 1..56: note = pUC-3'DB primer_F for preparing DB-M1
  source 1..56: mol_type = other DNA
taatacgactcactatagggagaccctcaaaaatcgagggtctcccctagttgttg

SEQ ID NO: 10 - DNA, 31 bp, synthetic construct
  misc_feature 1..31: note = pUC-3'DB primer_R for preparing DB-M1
  source 1..31: mol_type = other DNA
ctagttgttgtgtggaattgtcgacttttgt

SEQ ID NO: 11 - DNA, 53 bp, synthetic construct
  misc_feature 1..53: note = pUC-3'DB primer_F for preparing DB-M2
  source 1..53: mol_type = other DNA
taatacgactcactatagggagaccaaaaatcgagggtctcccctagttgttg

SEQ ID NO: 12 - DNA, 31 bp, synthetic construct; identical to SEQ ID NO: 10
  misc_feature 1..31: note = pUC-3'DB primer_R for preparing DB-M2
  source 1..31: mol_type = other DNA

SEQ ID NO: 13 - DNA, 50 bp, synthetic construct
  misc_feature 1..50: note = pUC-3'DB primer_F for preparing DB-M3
  source 1..50: mol_type = other DNA
taatacgactcactatagggagaaaaatcgagggcctcccctagttgttg

SEQ ID NO: 14 - DNA, 31 bp, synthetic construct; identical to SEQ ID NO: 10
  misc_feature 1..31: note = pUC-3'DB primer_R for preparing DB-M3
  source 1..31: mol_type = other DNA

SEQ ID NO: 15 - DNA, 84 bp, synthetic construct
  misc_feature 1..84: note = primer_F for preparing 271nt DNA template
  source 1..84: mol_type = other DNA
ccataatacgactcactatagggagaaaaatcgagggcctcccctagttgttgtgtggaattatggacagcaaaggttcgtcgc

SEQ ID NO: 16 - DNA, 41 bp, synthetic construct
  misc_feature 1..41: note = primer_R for preparing 271nt DNA template
  source 1..41: mol_type = other DNA
ctagttgttgtgtggaattttagaactccagggggaaggcc

SEQ ID NO: 17 - DNA, 94 bp, synthetic construct
  misc_feature 1..94: note = primer_F for preparing 997nt DNA template
  source 1..94: mol_type = other DNA
ccataatacgactcactatagggagaaaaatcgagggcctcccctagttgttgtgtggaattatgacttcgaaagtttatgatccagaacaaag

SEQ ID NO: 18 - DNA, 53 bp, synthetic construct
  misc_feature 1..53: note = primer_R for preparing 997nt DNA template
  source 1..53: mol_type = other DNA
ctagttgttgtgtggaattttattgttcatttttgagaactcgctcaacgaac

SEQ ID NO: 19 - DNA, 82 bp, synthetic construct
  misc_feature 1..82: note = primer_F for preparing 2308nt DNA template
  source 1..82: mol_type = other DNA
ccataatacgactcactatagggagaaaaatcgagggcctcccctagttgttgtgtggaattatggccttaccagtgaccgc

SEQ ID NO: 20 - DNA, 44 bp, synthetic construct
  misc_feature 1..44: note = primer_R for preparing 2308nt DNA template
  source 1..44: mol_type = other DNA
ctagttgttgtgtggaattttacttgtacagctcgtccatgccg

SEQ ID NO: 21 - DNA, 96 bp, synthetic construct
  misc_feature 1..96: note = primer_F for preparing 3004nt DNA template
  source 1..96: mol_type = other DNA
ccataatacgactcactatagggagaaaaatcgagggcctcccctagttgttgtgtggaattatgtcttattctgatgagtctcgactgtcgaatc

SEQ ID NO: 22 - DNA, 49 bp, synthetic construct
  misc_feature 1..49: note = primer_R for preparing 3004nt DNA template
  source 1..49: mol_type = other DNA
ctagttgttgtgtggaattttacttttcaaacctcccttcagcctgttg

SEQ ID NO: 23 - DNA, 96 bp, synthetic construct; identical to SEQ ID NO: 21
  misc_feature 1..96: note = primer_F for preparing 4000nt DNA template
  source 1..96: mol_type = other DNA

SEQ ID NO: 24 - DNA, 44 bp, synthetic construct
  misc_feature 1..44: note = primer_R for preparing 4000nt DNA template
  source 1..44: mol_type = other DNA
ctagttgttgtgtggaattttactgaacttcactgcactgtgcc

SEQ ID NO: 25 - DNA, 96 bp, synthetic construct; identical to SEQ ID NO: 21
  misc_feature 1..96: note = primer_F for preparing 5002nt DNA template
  source 1..96: mol_type = other DNA

SEQ ID NO: 26 - DNA, 50 bp, synthetic construct
  misc_feature 1..50: note = primer_R for preparing 5002nt DNA template
  source 1..50: mol_type = other DNA
ctagttgttgtgtggaattttacacaatcatgtcatcagtgctctgttcc

SEQ ID NO: 27 - DNA, 30 bp, synthetic construct
  misc_feature 1..30: note = DNA splint_30nt
  source 1..30: mol_type = other DNA
ctcgatttttctcccgtcgacttttgtttt

SEQ ID NO: 28 - DNA, 60 bp, synthetic construct
  misc_feature 1..60: note = DNA splint_60nt
  source 1..60: mol_type = other DNA
caactaggggagaccctcgatttttctcccgtcgacttttgttttttgttttttttttgt

SEQ ID NO: 29 - DNA, 91 bp, synthetic construct
  misc_feature 1..91: note = DNA splint_90nt
  source 1..91: mol_type = other DNA
gtaattccacacaacaactaggggagaccctcgatttttctcccgtcgacttttgttttttgttttttttttgttttttgttttttttttg

SEQ ID NO: 30 - DNA, 1844 bp, synthetic construct
  misc_feature 1..1844: note = DB-WT(13 nt + 19 nt double strand)
  source 1..1844: mol_type = other DNA
gggagaccctcgaaaaaatcgagggtctcccctagttgttgtgtggaattacaaaacacagcggccgcttaaaacagcctgtgggttgatcccacccacaggcccattgggcgctagcactctggtatcacggtacctttgtgcgcctgttttataccccctcccccaactgtaacttagaagtaacacacaccgatcaacagtcagcgtggcacaccagccacgttttgatcaagcacttctgttaccccggactgagtatcaatagactgctcacgcggttgaaggagaaagcgttcgttatccggccaactacttcgaaaaacctagtaacaccgtggaagttgcagagtgtttcgctcagcactaccccagtgtagatcaggtcgatgagtcaccgcattccccacgggcgaccgtggcggtggctgcgttggcggcctgcccatggggaaacccatgggacgctctaatacagacatggtgcgaagagtctattgagctagttggtagtcctccggcccctgaatgcggctaatcctaactgcggagcacacaccctcaagccagagggcagtgtgtcgtaacgggcaactctgcagcggaaccgactactttgggtgtccgtgtttcattttattcctatactggctgcttatggtgacaattgagagatcgttaccatatagctattggattggccatccggtgactaatagagctattatatatccctttgttgggtttataccacttagcttgaaagaggttaaaacattacaattcattgttaagttgaatacagcaaaatgggcgatcgcatgacttcgaaagtttatgatccagaacaaaggaaacggatgataactggtccgcagtggtgggccagatgtaaacaaatgaatgttcttgattcatttattaattattatgattcagaaaaacatgcagaaaatgctgttatttttttacatggtaacgcggcctcttcttatttatggcgacatgttgtgccacatattgagccagtagcgcggtgtattataccagaccttattggtatgggcaaatcaggcaaatctggtaatggttcttataggttacttgatcattacaaatatcttactgcatggtttgaacttcttaatttaccaaagaagatcatttttgtcggccatgattggggtgcttgtttggcatttcattatagctatgagcatcaagataagatcaaagcaatagttcacgctgaaagtgtagtagatgtgattgaatcatgggatgaatggcctgatattgaagaagatattgcgttgatcaaatctgaagaaggagaaaaaatggttttggagaataacttcttcgtggaaaccatgttgccatcaaaaatcatgagaaagttagaaccagaagaatttgcagcatatcttgaaccattcaaagagaaaggtgaagttcgtcgtccaacattatcatggcctcgtgaaatcccgttagtaaaaggtggtaaacctgacgttgtacaaattgttaggaattataatgcttatctacgtgcaagtgatgatttaccaaaaatgtttattgaatcggacccaggattcttttccaatgctattgttgaaggtgccaagaagtttcctaatactgaatttgtcaaagtaaaaggtcttcatttttcgcaagaagatgcacctgatgaaatgggaaaatatatcaaatcgttcgttgagcgagttctcaaaaatgaacaataaggcgcgccaaaaaacaaaaaacaaaaaaaaaacaaaaaacaaaaaaaaaacaaaaaacaaaagtcgacaattccacacaacaactag

SEQ ID NO: 31 - DNA, 1834 bp, synthetic construct
  misc_feature 1..1834: note = 3'DB
  source 1..1834: mol_type = other DNA
ggaaaaaatcgagggtctcccctagttgttgtgtggaattacaaaacacagcggccgcttaaaacagcctgtgggttgatcccacccacaggcccattgggcgctagcactctggtatcacggtacctttgtgcgcctgttttataccccctcccccaactgtaacttagaagtaacacacaccgatcaacagtcagcgtggcacaccagccacgttttgatcaagcacttctgttaccccggactgagtatcaatagactgctcacgcggttgaaggagaaagcgttcgttatccggccaactacttcgaaaaacctagtaacaccgtggaagttgcagagtgtttcgctcagcactaccccagtgtagatcaggtcgatgagtcaccgcattccccacgggcgaccgtggcggtggctgcgttggcggcctgcccatggggaaacccatgggacgctctaatacagacatggtgcgaagagtctattgagctagttggtagtcctccggcccctgaatgcggctaatcctaactgcggagcacacaccctcaagccagagggcagtgtgtcgtaacgggcaactctgcagcggaaccgactactttgggtgtccgtgtttcattttattcctatactggctgcttatggtgacaattgagagatcgttaccatatagctattggattggccatccggtgactaatagagctattatatatccctttgttgggtttataccacttagcttgaaagaggttaaaacattacaattcattgttaagttgaatacagcaaaatgggcgatcgcatgacttcgaaagtttatgatccagaacaaaggaaacggatgataactggtccgcagtggtgggccagatgtaaacaaatgaatgttcttgattcatttattaattattatgattcagaaaaacatgcagaaaatgctgttatttttttacatggtaacgcggcctcttcttatttatggcgacatgttgtgccacatattgagccagtagcgcggtgtattataccagaccttattggtatgggcaaatcaggcaaatctggtaatggttcttataggttacttgatcattacaaatatcttactgcatggtttgaacttcttaatttaccaaagaagatcatttttgtcggccatgattggggtgcttgtttggcatttcattatagctatgagcatcaagataagatcaaagcaatagttcacgctgaaagtgtagtagatgtgattgaatcatgggatgaatggcctgatattgaagaagatattgcgttgatcaaatctgaagaaggagaaaaaatggttttggagaataacttcttcgtggaaaccatgttgccatcaaaaatcatgagaaagttagaaccagaagaatttgcagcatatcttgaaccattcaaagagaaaggtgaagttcgtcgtccaacattatcatggcctcgtgaaatcccgttagtaaaaggtggtaaacctgacgttgtacaaattgttaggaattataatgcttatctacgtgcaagtgatgatttaccaaaaatgtttattgaatcggacccaggattcttttccaatgctattgttgaaggtgccaagaagtttcctaatactgaatttgtcaaagtaaaaggtcttcatttttcgcaagaagatgcacctgatgaaatgggaaaatatatcaaatcgttcgttgagcgagttctcaaaaatgaacaataaggcgcgccaaaaaacaaaaaacaaaaaaaaaacaaaaaacaaaaaaaaaacaaaaaacaaaagtcgacaattccacacaacaactag

SEQ ID NO: 32 - DNA, 1825 bp, synthetic construct
  misc_feature 1..1825: note = 5'DB
  source 1..1825: mol_type = other DNA
gggagaccctcgaaaaaatcgagggtctcccctagttgttgtgtggaattacaaaacacagcggccgcttaaaacagcctgtgggttgatcccacccacaggcccattgggcgctagcactctggtatcacggtacctttgtgcgcctgttttataccccctcccccaactgtaacttagaagtaacacacaccgatcaacagtcagcgtggcacaccagccacgttttgatcaagcacttctgttaccccggactgagtatcaatagactgctcacgcggttgaaggagaaagcgttcgttatccggccaactacttcgaaaaacctagtaacaccgtggaagttgcagagtgtttcgctcagcactaccccagtgtagatcaggtcgatgagtcaccgcattccccacgggcgaccgtggcggtggctgcgttggcggcctgcccatggggaaacccatgggacgctctaatacagacatggtgcgaagagtctattgagctagttggtagtcctccggcccctgaatgcggctaatcctaactgcggagcacacaccctcaagccagagggcagtgtgtcgtaacgggcaactctgcagcggaaccgactactttgggtgtccgtgtttcattttattcctatactggctgcttatggtgacaattgagagatcgttaccatatagctattggattggccatccggtgactaatagagctattatatatccctttgttgggtttataccacttagcttgaaagaggttaaaacattacaattcattgttaagttgaatacagcaaaatgggcgatcgcatgacttcgaaagtttatgatccagaacaaaggaaacggatgataactggtccgcagtggtgggccagatgtaaacaaatgaatgttcttgattcatttattaattattatgattcagaaaaacatgcagaaaatgctgttatttttttacatggtaacgcggcctcttcttatttatggcgacatgttgtgccacatattgagccagtagcgcggtgtattataccagaccttattggtatgggcaaatcaggcaaatctggtaatggttcttataggttacttgatcattacaaatatcttactgcatggtttgaacttcttaatttaccaaagaagatcatttttgtcggccatgattggggtgcttgtttggcatttcattatagctatgagcatcaagataagatcaaagcaatagttcacgctgaaagtgtagtagatgtgattgaatcatgggatgaatggcctgatattgaagaagatattgcgttgatcaaatctgaagaaggagaaaaaatggttttggagaataacttcttcgtggaaaccatgttgccatcaaaaatcatgagaaagttagaaccagaagaatttgcagcatatcttgaaccattcaaagagaaaggtgaagttcgtcgtccaacattatcatggcctcgtgaaatcccgttagtaaaaggtggtaaacctgacgttgtacaaattgttaggaattataatgcttatctacgtgcaagtgatgatttaccaaaaatgtttattgaatcggacccaggattcttttccaatgctattgttgaaggtgccaagaagtttcctaatactgaatttgtcaaagtaaaaggtcttcatttttcgcaagaagatgcacctgatgaaatgggaaaatatatcaaatcgttcgttgagcgagttctcaaaaatgaacaataaggcgcgccaaaaaacaaaaaacaaaaaaaaaacaaaaaacaaaaaaaaaacaaaaaacaaaagtcgac

SEQ ID NO: 33 - DNA, 1815 bp, synthetic construct
  misc_feature 1..1815: note = 5' and 3' DB deletion
  source 1..1815: mol_type = other DNA
ggaaaaaatcgagggtctcccctagttgttgtgtggaattacaaaacacagcggccgcttaaaacagcctgtgggttgatcccacccacaggcccattgggcgctagcactctggtatcacggtacctttgtgcgcctgttttataccccctcccccaactgtaacttagaagtaacacacaccgatcaacagtcagcgtggcacaccagccacgttttgatcaagcacttctgttaccccggactgagtatcaatagactgctcacgcggttgaaggagaaagcgttcgttatccggccaactacttcgaaaaacctagtaacaccgtggaagttgcagagtgtttcgctcagcactaccccagtgtagatcaggtcgatgagtcaccgcattccccacgggcgaccgtggcggtggctgcgttggcggcctgcccatggggaaacccatgggacgctctaatacagacatggtgcgaagagtctattgagctagttggtagtcctccggcccctgaatgcggctaatcctaactgcggagcacacaccctcaagccagagggcagtgtgtcgtaacgggcaactctgcagcggaaccgactactttgggtgtccgtgtttcattttattcctatactggctgcttatggtgacaattgagagatcgttaccatatagctattggattggccatccggtgactaatagagctattatatatccctttgttgggtttataccacttagcttgaaagaggttaaaacattacaattcattgttaagttgaatacagcaaaatgggcgatcgcatgacttcgaaagtttatgatccagaacaaaggaaacggatgataactggtccgcagtggtgggccagatgtaaacaaatgaatgttcttgattcatttattaattattatgattcagaaaaacatgcagaaaatgctgttatttttttacatggtaacgcggcctcttcttatttatggcgacatgttgtgccacatattgagccagtagcgcggtgtattataccagaccttattggtatgggcaaatcaggcaaatctggtaatggttcttataggttacttgatcattacaaatatcttactgcatggtttgaacttcttaatttaccaaagaagatcatttttgtcggccatgattggggtgcttgtttggcatttcattatagctatgagcatcaagataagatcaaagcaatagttcacgctgaaagtgtagtagatgtgattgaatcatgggatgaatggcctgatattgaagaagatattgcgttgatcaaatctgaagaaggagaaaaaatggttttggagaataacttcttcgtggaaaccatgttgccatcaaaaatcatgagaaagttagaaccagaagaatttgcagcatatcttgaaccattcaaagagaaaggtgaagttcgtcgtccaacattatcatggcctcgtgaaatcccgttagtaaaaggtggtaaacctgacgttgtacaaattgttaggaattataatgcttatctacgtgcaagtgatgatttaccaaaaatgtttattgaatcggacccaggattcttttccaatgctattgttgaaggtgccaagaagtttcctaatactgaatttgtcaaagtaaaaggtcttcatttttcgcaagaagatgcacctgatgaaatgggaaaatatatcaaatcgttcgttgagcgagttctcaaaaatgaacaataaggcgcgccaaaaaacaaaaaacaaaaaaaaaacaaaaaacaaaaaaaaaacaaaaaacaaaagtcgac

SEQ ID NO: 34 - DNA, 1815 bp, synthetic construct
  misc_feature 1..1815: note = 3'DB-M1
  source 1..1815: mol_type = other DNA
ggaaaaatccctagttgttgtgtggacaaaacacagcggccgcttaaaacagcctgtgggttgatcccacccacaggcccattgggcgctagcactctggtatcacggtacctttgtgcgcctgttttataccccctcccccaactgtaacttagaagtaacacacaccgatcaacagtcagcgtggcacaccagccacgttttgatcaagcacttctgttaccccggactgagtatcaatagactgctcacgcggttgaaggagaaagcgttcgttatccggccaactacttcgaaaaacctagtaacaccgtggaagttgcagagtgtttcgctcagcactaccccagtgtagatcaggtcgatgagtcaccgcattccccacgggcgaccgtggcggtggctgcgttggcggcctgcccatggggaaacccatgggacgctctaatacagacatggtgcgaagagtctattgagctagttggtagtcctccggcccctgaatgcggctaatcctaactgcggagcacacaccctcaagccagagggcagtgtgtcgtaacgggcaactctgcagcggaaccgactactttgggtgtccgtgtttcattttattcctatactggctgcttatggtgacaattgagagatcgttaccatatagctattggattggccatccggtgactaatagagctattatatatccctttgttgggtttataccacttagcttgaaagaggttaaaacattacaattcattgttaagttgaatacagcaaaatgggcgatcgcatgacttcgaaagtttatgatccagaacaaaggaaacggatgataactggtccgcagtggtgggccagatgtaaacaaatgaatgttcttgattcatttattaattattatgattcagaaaaacatgcagaaaatgctgttatttttttacatggtaacgcggcctcttcttatttatggcgacatgttgtgccacatattgagccagtagcgcggtgtattataccagaccttattggtatgggcaaatcaggcaaatctggtaatggttcttataggttacttgatcattacaaatatcttactgcatggtttgaacttcttaatttaccaaagaagatcatttttgtcggccatgattggggtgcttgtttggcatttcattatagctatgagcatcaagataagatcaaagcaatagttcacgctgaaagtgtagtagatgtgattgaatcatgggatgaatggcctgatattgaagaagatattgcgttgatcaaatctgaagaaggagaaaaaatggttttggagaataacttcttcgtggaaaccatgttgccatcaaaaatcatgagaaagttagaaccagaagaatttgcagcatatcttgaaccattcaaagagaaaggtgaagttcgtcgtccaacattatcatggcctcgtgaaatcccgttagtaaaaggtggtaaacctgacgttgtacaaattgttaggaattataatgcttatctacgtgcaagtgatgatttaccaaaaatgtttattgaatcggacccaggattcttttccaatgctattgttgaaggtgccaagaagtttcctaatactgaatttgtcaaagtaaaaggtcttcatttttcgcaagaagatgcacctgatgaaatgggaaaatatatcaaatcgttcgttgagcgagttctcaaaaatgaacaataaggcgcgccaaaaaacaaaaaacaaaaaaaaaacaaaaaacaaaaaaaaaacaaaaaacaaaagtcgacccacacaacaactag

SEQ ID NO: 35 - DNA, 1805 bp, synthetic construct
  misc_feature 1..1805: note = 3'DB-M2
  source 1..1805: mol_type = other DNA
ggaaaaatccctagttgtggacaaaacacagcggccgcttaaaacagcctgtgggttgatcccacccacaggcccattgggcgctagcactctggtatcacggtacctttgtgcgcctgttttataccccctcccccaactgtaacttagaagtaacacacaccgatcaacagtcagcgtggcacaccagccacgttttgatcaagcacttctgttaccccggactgagtatcaatagactgctcacgcggttgaaggagaaagcgttcgttatccggccaactacttcgaaaaacctagtaacaccgtggaagttgcagagtgtttcgctcagcactaccccagtgtagatcaggtcgatgagtcaccgcattccccacgggcgaccgtggcggtggctgcgttggcggcctgcccatggggaaacccatgggacgctctaatacagacatggtgcgaagagtctattgagctagttggtagtcctccggcccctgaatgcggctaatcctaactgcggagcacacaccctcaagccagagggcagtgtgtcgtaacgggcaactctgcagcggaaccgactactttgggtgtccgtgtttcattttattcctatactggctgcttatggtgacaattgagagatcgttaccatatagctattggattggccatccggtgactaatagagctattatatatccctttgttgggtttataccacttagcttgaaagaggttaaaacattacaattcattgttaagttgaatacagcaaaatgggcgatcgcatgacttcgaaagtttatgatccagaacaaaggaaacggatgataactggtccgcagtggtgggccagatgtaaacaaatgaatgttcttgattcatttattaattattatgattcagaaaaacatgcagaaaatgctgttatttttttacatggtaacgcggcctcttcttatttatggcgacatgttgtgccacatattgagccagtagcgcggtgtattataccagaccttattggtatgggcaaatcaggcaaatctggtaatggttcttataggttacttgatcattacaaatatcttactgcatggtttgaacttcttaatttaccaaagaagatcatttttgtcggccatgattggggtgcttgtttggcatttcattatagctatgagcatcaagataagatcaaagcaatagttcacgctgaaagtgtagtagatgtgattgaatcatgggatgaatggcctgatattgaagaagatattgcgttgatcaaatctgaagaaggagaaaaaatggttttggagaataacttcttcgtggaaaccatgttgccatcaaaaatcatgagaaagttagaaccagaagaatttgcagcatatcttgaaccattcaaagagaaaggtgaagttcgtcgtccaacattatcatggcctcgtgaaatcccgttagtaaaaggtggtaaacctgacgttgtacaaattgttaggaattataatgcttatctacgtgcaagtgatgatttaccaaaaatgtttattgaatcggacccaggattcttttccaatgctattgttgaaggtgccaagaagtttcctaatactgaatttgtcaaagtaaaaggtcttcatttttcgcaagaagatgcacctgatgaaatgggaaaatatatcaaatcgttcgttgagcgagttctcaaaaatgaacaataaggcgcgccaaaaaacaaaaaacaaaaaaaaaacaaaaaacaaaaaaaaaacaaaaaacaaaagtcgacccacaactag

SEQ ID NO: 36 - DNA, 1805 bp, synthetic construct
  misc_feature 1..1805: note = 3'DB-M3
  source 1..1805: mol_type = other DNA
ggaaaaatccctagtcgcggacaaaacacagcggccgcttaaaacagcctgtgggttgatcccacccacaggcccattgggcgctagcactctggtatcacggtacctttgtgcgcctgttttataccccctcccccaactgtaacttagaagtaacacacaccgatcaacagtcagcgtggcacaccagccacgttttgatcaagcacttctgttaccccggactgagtatcaatagactgctcacgcggttgaaggagaaagcgttcgttatccggccaactacttcgaaaaacctagtaacaccgtggaagttgcagagtgtttcgctcagcactaccccagtgtagatcaggtcgatgagtcaccgcattccccacgggcgaccgtggcggtggctgcgttggcggcctgcccatggggaaacccatgggacgctctaatacagacatggtgcgaagagtctattgagctagttggtagtcctccggcccctgaatgcggctaatcctaactgcggagcacacaccctcaagccagagggcagtgtgtcgtaacgggcaactctgcagcggaaccgactactttgggtgtccgtgtttcattttattcctatactggctgcttatggtgacaattgagagatcgttaccatatagctattggattggccatccggtgactaatagagctattatatatccctttgttgggtttataccacttagcttgaaagaggttaaaacattacaattcattgttaagttgaatacagcaaaatgggcgatcgcatgacttcgaaagtttatgatccagaacaaaggaaacggatgataactggtccgcagtggtgggccagatgtaaacaaatgaatgttcttgattcatttattaattattatgattcagaaaaacatgcagaaaatgctgttatttttttacatggtaacgcggcctcttcttatttatggcgacatgttgtgccacatattgagccagtagcgcggtgtattataccagaccttattggtatgggcaaatcaggcaaatctggtaatggttcttataggttacttgatcattacaaatatcttactgcatggtttgaacttcttaatttaccaaagaagatcatttttgtcggccatgattggggtgcttgtttggcatttcattatagctatgagcatcaagataagatcaaagcaatagttcacgctgaaagtgtagtagatgtgattgaatcatgggatgaatggcctgatattgaagaagatattgcgttgatcaaatctgaagaaggagaaaaaatggttttggagaataacttcttcgtggaaaccatgttgccatcaaaaatcatgagaaagttagaaccagaagaatttgcagcatatcttgaaccattcaaagagaaaggtgaagttcgtcgtccaacattatcatggcctcgtgaaatcccgttagtaaaaggtggtaaacctgacgttgtacaaattgttaggaattataatgcttatctacgtgcaagtgatgatttaccaaaaatgtttattgaatcggacccaggattcttttccaatgctattgttgaaggtgccaagaagtttcctaatactgaatttgtcaaagtaaaaggtcttcatttttcgcaagaagatgcacctgatgaaatgggaaaatatatcaaatcgttcgttgagcgagttctcaaaaatgaacaataaggcgcgccaaaaaacaaaaaacaaaaaaaaaacaaaaaacaaaaaaaaaacaaaaaacaaaagtcgacccgcgactag

SEQ ID NO: 37 - DNA, 1842 bp, synthetic construct
  misc_feature 1..1842: note = "DB-M1 (11 nt + 19 nt double strand RNA)"
  source 1..1842: mol_type = other DNA
gggagaccctcaaaaatcgagggtctcccctagttgttgtgtggaattacaaaacacagcggccgcttaaaacagcctgtgggttgatcccacccacaggcccattgggcgctagcactctggtatcacggtacctttgtgcgcctgttttataccccctcccccaactgtaacttagaagtaacacacaccgatcaacagtcagcgtggcacaccagccacgttttgatcaagcacttctgttaccccggactgagtatcaatagactgctcacgcggttgaaggagaaagcgttcgttatccggccaactacttcgaaaaacctagtaacaccgtggaagttgcagagtgtttcgctcagcactaccccagtgtagatcaggtcgatgagtcaccgcattccccacgggcgaccgtggcggtggctgcgttggcggcctgcccatggggaaacccatgggacgctctaatacagacatggtgcgaagagtctattgagctagttggtagtcctccggcccctgaatgcggctaatcctaactgcggagcacacaccctcaagccagagggcagtgtgtcgtaacgggcaactctgcagcggaaccgactactttgggtgtccgtgtttcattttattcctatactggctgcttatggtgacaattgagagatcgttaccatatagctattggattggccatccggtgactaatagagctattatatatccctttgttgggtttataccacttagcttgaaagaggttaaaacattacaattcattgttaagttgaatacagcaaaatgggcgatcgcatgacttcgaaagtttatgatccagaacaaaggaaacggatgataactggtccgcagtggtgggccagatgtaaacaaatgaatgttcttgattcatttattaattattatgattcagaaaaacatgcagaaaatgctgttatttttttacatggtaacgcggcctcttcttatttatggcgacatgttgtgccacatattgagccagtagcgcggtgtattataccagaccttattggtatgggcaaatcaggcaaatctggtaatggttcttataggttacttgatcattacaaatatcttactgcatggtttgaacttcttaatttaccaaagaagatcatttttgtcggccatgattggggtgcttgtttggcatttcattatagctatgagcatcaagataagatcaaagcaatagttcacgctgaaagtgtagtagatgtgattgaatcatgggatgaatggcctgatattgaagaagatattgcgttgatcaaatctgaagaaggagaaaaaatggttttggagaataacttcttcgtggaaaccatgttgccatcaaaaatcatgagaaagttagaaccagaagaatttgcagcatatcttgaaccattcaaagagaaaggtgaagttcgtcgtccaacattatcatggcctcgtgaaatcccgttagtaaaaggtggtaaacctgacgttgtacaaattgttaggaattataatgcttatctacgtgcaagtgatgatttaccaaaaatgtttattgaatcggacccaggattcttttccaatgctattgttgaaggtgccaagaagtttcctaatactgaatttgtcaaagtaaaaggtcttcatttttcgcaagaagatgcacctgatgaaatgggaaaatatatcaaatcgttcgttgagcgagttctcaaaaatgaacaataaggcgcgccaaaaaacaaaaaacaaaaaaaaaacaaaaaacaaaaaaaaaacaaaaaacaaaagtcgacaattccacacaacaactag

SEQ ID NO: 38 - DNA, 1839 bp, synthetic construct
  misc_feature 1..1839: note = "DB-M2 (8 nt + 19 nt double strand RNA)"
  source 1..1839: mol_type = other DNA
gggagaccaaaaatcgagggtctcccctagttgttgtgtggaattacaaaacacagcggccgcttaaaacagcctgtgggttgatcccacccacaggcccattgggcgctagcactctggtatcacggtacctttgtgcgcctgttttataccccctcccccaactgtaacttagaagtaacacacaccgatcaacagtcagcgtggcacaccagccacgttttgatcaagcacttctgttaccccggactgagtatcaatagactgctcacgcggttgaaggagaaagcgttcgttatccggccaactacttcgaaaaacctagtaacaccgtggaagttgcagagtgtttcgctcagcactaccccagtgtagatcaggtcgatgagtcaccgcattccccacgggcgaccgtggcggtggctgcgttggcggcctgcccatggggaaacccatgggacgctctaatacagacatggtgcgaagagtctattgagctagttggtagtcctccggcccctgaatgcggctaatcctaactgcggagcacacaccctcaagccagagggcagtgtgtcgtaacgggcaactctgcagcggaaccgactactttgggtgtccgtgtttcattttattcctatactggctgcttatggtgacaattgagagatcgttaccatatagctattggattggccatccggtgactaatagagctattatatatccctttgttgggtttataccacttagcttgaaagaggttaaaacattacaattcattgttaagttgaatacagcaaaatgggcgatcgcatgacttcgaaagtttatgatccagaacaaaggaaacggatgataactggtccgcagtggtgggccagatgtaaacaaatgaatgttcttgattcatttattaattattatgattcagaaaaacatgcagaaaatgctgttatttttttacatggtaacgcggcctcttcttatttatggcgacatgttgtgccacatattgagccagtagcgcggtgtattataccagaccttattggtatgggcaaatcaggcaaatctggtaatggttcttataggttacttgatcattacaaatatcttactgcatggtttgaacttcttaatttaccaaagaagatcatttttgtcggccatgattggggtgcttgtttggcatttcattatagctatgagcatcaagataagatcaaagcaatagttcacgctgaaagtgtagtagatgtgattgaatcatgggatgaatggcctgatattgaagaagatattgcgttgatcaaatctgaagaaggagaaaaaatggttttggagaataacttcttcgtggaaaccatgttgccatcaaaaatcatgagaaagttagaaccagaagaatttgcagcatatcttgaaccattcaaagagaaaggtgaagttcgtcgtccaacattatcatggcctcgtgaaatcccgttagtaaaaggtggtaaacctgacgttgtacaaattgttaggaattataatgcttatctacgtgcaagtgatgatttaccaaaaatgtttattgaatcggacccaggattcttttccaatgctattgttgaaggtgccaagaagtttcctaatactgaatttgtcaaagtaaaaggtcttcatttttcgcaagaagatgcacctgatgaaatgggaaaatatatcaaatcgttcgttgagcgagttctcaaaaatgaacaataaggcgcgccaaaaaacaaaaaacaaaaaaaaaacaaaaaacaaaaaaaaaacaaaaaacaaaagtcgacaattccacacaacaactag

SEQ ID NO: 39 - DNA, 1836 bp, synthetic construct
  misc_feature 1..1836: note = "DB-M3 (5 nt + 19 nt double strand RNA)"
  source 1..1836: mol_type = other DNA
gggagaaaaatcgagggcctcccctagttgttgtgtggaattacaaaacacagcggccgcttaaaacagcctgtgggttgatcccacccacaggcccattgggcgctagcactctggtatcacggtacctttgtgcgcctgttttataccccctcccccaactgtaacttagaagtaacacacaccgatcaacagtcagcgtggcacaccagccacgttttgatcaagcacttctgttaccccggactgagtatcaatagactgctcacgcggttgaaggagaaagcgttcgttatccggccaactacttcgaaaaacctagtaacaccgtggaagttgcagagtgtttcgctcagcactaccccagtgtagatcaggtcgatgagtcaccgcattccccacgggcgaccgtggcggtggctgcgttggcggcctgcccatggggaaacccatgggacgctctaatacagacatggtgcgaagagtctattgagctagttggtagtcctccggcccctgaatgcggctaatcctaactgcggagcacacaccctcaagccagagggcagtgtgtcgtaacgggcaactctgcagcggaaccgactactttgggtgtccgtgtttcattttattcctatactggctgcttatggtgacaattgagagatcgttaccatatagctattggattggccatccggtgactaatagagctattatatatccctttgttgggtttataccacttagcttgaaagaggttaaaacattacaattcattgttaagttgaatacagcaaaatgggcgatcgcatgacttcgaaagtttatgatccagaacaaaggaaacggatgataactggtccgcagtggtgggccagatgtaaacaaatgaatgttcttgattcatttattaattattatgattcagaaaaacatgcagaaaatgctgttatttttttacatggtaacgcggcctcttcttatttatggcgacatgttgtgccacatattgagccagtagcgcggtgtattataccagaccttattggtatgggcaaatcaggcaaatctggtaatggttcttataggttacttgatcattacaaatatcttactgcatggtttgaacttcttaatttaccaaagaagatcatttttgtcggccatgattggggtgcttgtttggcatttcattatagctatgagcatcaagataagatcaaagcaatagttcacgctgaaagtgtagtagatgtgattgaatcatgggatgaatggcctgatattgaagaagatattgcgttgatcaaatctgaagaaggagaaaaaatggttttggagaataacttcttcgtggaaaccatgttgccatcaaaaatcatgagaaagttagaaccagaagaatttgcagcatatcttgaaccattcaaagagaaaggtgaagttcgtcgtccaacattatcatggcctcgtgaaatcccgttagtaaaaggtggtaaacctgacgttgtacaaattgttaggaattataatgcttatctacgtgcaagtgatgatttaccaaaaatgtttattgaatcggacccaggattcttttccaatgctattgttgaaggtgccaagaagtttcctaatactgaatttgtcaaagtaaaaggtcttcatttttcgcaagaagatgcacctgatgaaatgggaaaatatatcaaatcgttcgttgagcgagttctcaaaaatgaacaataaggcgcgccaaaaaacaaaaaacaaaaaaaaaacaaaaaacaaaaaaaaaacaaaaaacaaaagtcgacaattccacacaacaactag

SEQ ID NO: 40 - DNA, 288 bp, synthetic construct
  misc_feature 1..288: note = 271 nt DNA product
  source 1..288: mol_type = other DNA
ccataatacgactcactatagggagaaaaatcgagggcctcccctagttgttgtgtggaattgacagcaaaggttcgtcgcagaaagggtcccgcctgctcctgctgctggtggtgtcaaatctactcttgtgccagggtgtggtctcctcctactccatggagcacttccgctggggcaagccggtgggcaagaagcggcgcccagtgaaggtgtaccctaacggcgccgaggacgagtcggccgaggccttccccctggagttctaaaattccacacaacaactag

SEQ ID NO: 41 - DNA, 1017 bp, synthetic construct
  misc_feature 1..1017: note = 997 nt DNA product
  source 1..1017: mol_type = other DNA
ccataatacgactcactatagggagaaaaatcgagggcctcccctagttgttgtgtggaattatgacttcgaaagtttatgatccagaacaaaggaaacggatgataactggtccgcagtggtgggccagatgtaaacaaatgaatgttcttgattcatttattaattattatgattcagaaaaacatgcagaaaatgctgttatttttttacatggtaacgcggcctcttcttatttatggcgacatgttgtgccacatattgagccagtagcgcggtgtattataccagaccttattggtatgggcaaatcaggcaaatctggtaatggttcttataggttacttgatcattacaaatatcttactgcatggtttgaacttcttaatttaccaaagaagatcatttttgtcggccatgattggggtgcttgtttggcatttcattatagctatgagcatcaagataagatcaaagcaatagttcacgctgaaagtgtagtagatgtgattgaatcatgggatgaatggcctgatattgaagaagatattgcgttgatcaaatctgaagaaggagaaaaaatggttttggagaataacttcttcgtggaaaccatgttgccatcaaaaatcatgagaaagttagaaccagaagaatttgcagcatatcttgaaccattcaaagagaaaggtgaagttcgtcgtccaacattatcatggcctcgtgaaatcccgttagtaaaaggtggtaaacctgacgttgtacaaattgttaggaattataatgcttatctacgtgcaagtgatgatttaccaaaaatgtttattgaatcggacccaggattcttttccaatgctattgttgaaggtgccaagaagtttcctaatactgaatttgtcaaagtaaaaggtcttcatttttcgcaagaagatgcacctgatgaaatgggaaaatatatcaaatcgttcgttgagcgagttctcaaaaatgaacaataaaattccacacaacaactag

SEQ ID NO: 42 - DNA, 2328 bp, synthetic construct
  misc_feature 1..2328: note = 2300 nt DNA product
  source 1..2328: mol_type = other DNA
ccataatacgactcactatagggagaaaaatcgagggtctcccctagttgttgtgtggaattatggccttaccagtgaccgccttgctcctgccgctggccttgctgctccacgccgccaggccggacatccagatgacacagactacatcctccctgtctgcctctctgggagacagagtcaccatcagttgcagggcaagtcaggacattagtaaatatttaaattggtatcagcagaaaccagatggaactgttaaactcctgatctaccatacatcaagattacactcaggagtcccatcaaggttcagtggcagtgggtctggaacagattattctctcaccattagcaacctggagcaagaagatattgccacttacttttgccaacagggtaatacgcttccgtacacgttcggaggggggactaagttggaaataacaggtggcggtggctcgggcggtggtgggtcgggtggcggcggatctgaggtgaaactgcaggagtcaggacctggcctggtggcgccctcacagagcctgtccgtcacatgcactgtctcaggggtctcattacccgactatggtgtaagctggattcgccagcctccacgaaagggtctggagtggctgggagtaatatggggtagtgaaaccacatactataattcagctctcaaatccagactgaccatcatcaaggacaactccaagagccaagttttcttaaaaatgaacagtctgcaaactgatgacacagccatttactactgtgccaaacattattactacggtggtagctatgctatggactactggggtcaaggaacctcagtcaccgtctcctcaaccacgacgccagcgccgcgaccaccaacaccggcgcccaccatcgcgtcgcagcccctgtccctgcgcccagaggcgtgccggccagcggcggggggcgcagtgcacacgagggggctggacttcgcctgtgatatctacatctgggcgcccttggccgggacttgtggggtccttctcctgtcactggttatcaccctttactgcaaacggggcagaaagaaactcctgtatatattcaaacaaccatttatgagaccagtacaaactactcaagaggaagatggctgtagctgccgatttccagaagaagaagaaggaggatgtgaactgagagtgaagttcagcaggagcgcagacgcccccgcgtaccagcagggccagaaccagctctataacgagctcaatctaggacgaagagaggagtacgatgttttggacaagagacgtggccgggaccctgagatggggggaaagccgagaaggaagaaccctcaggaaggcctgtacaatgaactgcagaaagataagatggcggaggcctacagtgagattgggatgaaaggcgagcgccggaggggcaaggggcacgatggcctttaccagggtctcagtacagccaccaaggacacctacgacgcccttcacatgcaggccctgccccctcgcgaattcgagggcagaggaagtcttctaacatgcggtgacgtggaggagaatcccggccctggcgatcgcatggtgagcaagggcgaggagctgttcaccggggtggtgcccatcctggtcgagctggacggcgacgtaaacggccacaagttcagcgtgtccggcgagggcgagggcgatgccacctacggcaagctgaccctgaagttcatctgcaccaccggcaagctgcccgtgccctggcccaccctcgtgaccaccttcggctacggcctgcagtgcttcgcccgctaccccgaccacatgaagcagcacgacttcttcaagtccgccatgcccgaaggctacgtccaggagcgcaccatcttcttcaaggacgacggcaactacaagacccgcgccgaggtgaagttcgagggcgacaccctggtgaaccgcatcgagctgaagggcatcgacttcaaggaggacggcaacatcctggggcacaagctggagtacaactacaacagccacaacgtctatatcatggccgacaagcagaagaacggcatcaaggtgaacttcaagatccgccacaacatcgaggacggcagcgtgcagctcgccgaccactaccagcagaacacccccatcggcgacggccccgtgctgctgcccgacaaccactacctgagctaccagtccgccctgagcaaagaccccaacgagaagcgcgatcacatggtcctgctggagttcgtgaccgccgccgggatcactctcggcatggacgagctgtacaagtaaaattccacacaacaactag

SEQ ID NO: 43 - DNA, 3024 bp, synthetic construct
  misc_feature 1..3024: note = 3004 nt DNA product
  source 1..3024: mol_type = other DNA
caataatacgactcactatagggagaaaaatcgagggtctcccctagttgttgtgtggaattatgtcttattctgatgagtctcgactgtcgaatcttcttcggaggatcacccgggaagacgacagagaccgaagattggctactgtaaagcagttgaaagaatttattcagcaaccagaaaataagctggtactagttaaacaattggataatatcttggctgctgtacatgacgtgcttaatgaaagtagcaaattgcttcaggagttgagacaggagggagcttgctgtcttggccttctttgtgcttctctgagctatgaggctgagaagatcttcaagtggatttttagcaaatttagctcatctgcaaaagatgaagttaaactcctctacttatgtgccacctacaaagcactagagactgtaggagaaaagaaagccttttcatctgtaatgcagcttgtaatgaccagcctgcagtctattcttgaaaatgtggatacaccagaattgctttgtaaatgtgttaagtgcattcttttggtggctcgatgttaccctcatattttcagcactaattttagggatacagttgatatattagttggatggcatatagatcatactcagaaaccttcgctcacgcagcaggtatctgggtggttgcagagtttggagccattttgggtagctgatcttgcattttctactactcttcttggtcagtttctggaagacatggaagcatatgctgaggacctcagccatgtggcctctggggaatcagtggatgaagatgtccctcctccatcagtgtcattaccaaagctggctgcacttctccgggtatttagtactgtggtgaggagcattggggaacgcttcagcccaattcggggtcctccaattactgaggcatatgtaacagatgttctgtacagagtaatgagatgtgtgacggctgcaaaccaggtgtttttttctgaggctgtgttgacagctgctaatgagtgtgttggtgttttgctcggcagcttggatcctagcatgactatacattgtgacatggtcattacatatggattagaccaactggagaattgccagacttgtggtaccgattatatcatctcagtcttgaatttactcacgctgattgttgaacagataaatacgaaactgccatcatcatttgtagaaaaactgtttataccatcatctaaactactattcttgcgttatcataaagaaaaagaggttgttgctgtagcccatgctgtttatcaagcagtgctcagcttgaagaatattcctgttttggagactgcctataagttaatattgggagaaatgacttgtgccctaaacaacctcctacacagtctacaacttcctgaggcctgttctgaaataaaacatgaggcttttaagaatcatgtgttcaatgtagacaatgcaaaatttgtagttatatttgacctcagtgccctgactacaattggaaatgccaaaaactcactaatagggatgtgggcgctatctccaactgtctttgcacttctgagtaagaatctgatgattgtgcacagtgacctggctgttcacttccctgccattcagtatgctgtgctctacacattgtattctcattgtaccaggcatgatcactttatctctagtagcctcagttcttcctctccttctttgtttgatggagctgtgattagcactgtaactacggctacaaagaaacatttctcaattatattaaatcttctgggaatattacttaagaaagataaccttaaccaggacacgaggaaactgttaatgacttgggctttggaagcagctgttttaatgaagaagtctgaaacatacgcacctttattctctcttccgtctttccataaattttgcaaaggccttttagccaacactctcgttgaagatgtgaatatctgtctgcaggcatgcagcagtctacatgctctgtcctcttccttgccagatgatcttttacagagatgtgtcgatgtttgccgtgttcaactagtgcacagtggaactcgtattcgacaagcatttggaaaactgttgaaatcaattcctttagatgttgtcctaagcaataacaatcacacagaaattcaagaaatttctttagcattaagaagtcacatgagtaaagcaccaagtaatacattccacccccaagatttctctgatgttattagttttattttgtatgggaactctcatagaacagggaaggacaattggttggaaagactgttctatagctgccagagactggataagcgtgaccagtcaacaattccacgcaatctcctgaagacagatgctgtcctttggcagtgggccatatgggaagctgcacaattcactgttctttctaagctgagaaccccactgggcagagctcaagacaccttccagacaattgaaggtatcattcgaagtctcgcagctcacacattaaaccctgatcaggatgttagtcagtggacaactgcagacaatgatgaaggccatggtaacaaccaacttagacttgttcttcttctgcagtatctggaaaatctggagaaattaatgtataatgcatacgagggatgtgctaatgcattaacttcacctcccaaggtcattagaacttttttctataccaatcgccaaacttgtcaggactggctaacgcggattcgactctccatcatgagggtaggattgttggcaggccagcctgcagtgacagtgagacatggctttgacttgcttacagagatgaaaacaaccagcctatctcaggggaatgaattggaagtaaccattatgatggtggtagaagcattatgtgaacttcattgtcctgaagctatacagggaattgctgtctggtcatcatctattgttggaaaaaatcttctgtggattaactcagtggctcaacaggctgaagggaggtttgaaaagtaaaattccacacaacaactag

SEQ ID NO: 44 - DNA, 4000 bp, synthetic construct
  misc_feature 1..4000: note = 4000 nt DNA product
  source 1..4000: mol_type = other DNA
gggagaaaaatcgagggtctcccctagttgttgtgtggaattatgtcttattctgatgagtctcgactgtcgaatcttcttcggaggatcacccgggaagacgacagagaccgaagattggctactgtaaagcagttgaaagaatttattcagcaaccagaaaataagctggtactagttaaacaattggataatatcttggctgctgtacatgacgtgcttaatgaaagtagcaaattgcttcaggagttgagacaggagggagcttgctgtcttggccttctttgtgcttctctgagctatgaggctgagaagatcttcaagtggatttttagcaaatttagctcatctgcaaaagatgaagttaaactcctctacttatgtgccacctacaaagcactagagactgtaggagaaaagaaagccttttcatctgtaatgcagcttgtaatgaccagcctgcagtctattcttgaaaatgtggatacaccagaattgctttgtaaatgtgttaagtgcattcttttggtggctcgatgttaccctcatattttcagcactaattttagggatacagttgatatattagttggatggcatatagatcatactcagaaaccttcgctcacgcagcaggtatctgggtggttgcagagtttggagccattttgggtagctgatcttgcattttctactactcttcttggtcagtttctggaagacatggaagcatatgctgaggacctcagccatgtggcctctggggaatcagtggatgaagatgtccctcctccatcagtgtcattaccaaagctggctgcacttctccgggtatttagtactgtggtgaggagcattggggaacgcttcagcccaattcggggtcctccaattactgaggcatatgtaacagatgttctgtacagagtaatgagatgtgtgacggctgcaaaccaggtgtttttttctgaggctgtgttgacagctgctaatgagtgtgttggtgttttgctcggcagcttggatcctagcatgactatacattgtgacatggtcattacatatggattagaccaactggagaattgccagacttgtggtaccgattatatcatctcagtcttgaatttactcacgctgattgttgaacagataaatacgaaactgccatcatcatttgtagaaaaactgtttataccatcatctaaactactattcttgcgttatcataaagaaaaagaggttgttgctgtagcccatgctgtttatcaagcagtgctcagcttgaagaatattcctgttttggagactgcctataagttaatattgggagaaatgacttgtgccctaaacaacctcctacacagtctacaacttcctgaggcctgttctgaaataaaacatgaggcttttaagaatcatgtgttcaatgtagacaatgcaaaatttgtagttatatttgacctcagtgccctgactacaattggaaatgccaaaaactcactaatagggatgtgggcgctatctccaactgtctttgcacttctgagtaagaatctgatgattgtgcacagtgacctggctgttcacttccctgccattcagtatgctgtgctctacacattgtattctcattgtaccaggcatgatcactttatctctagtagcctcagttcttcctctccttctttgtttgatggagctgtgattagcactgtaactacggctacaaagaaacatttctcaattatattaaatcttctgggaatattacttaagaaagataaccttaaccaggacacgaggaaactgttaatgacttgggctttggaagcagctgttttaatgaagaagtctgaaacatacgcacctttattctctcttccgtctttccataaattttgcaaaggccttttagccaacactctcgttgaagatgtgaatatctgtctgcaggcatgcagcagtctacatgctctgtcctcttccttgccagatgatcttttacagagatgtgtcgatgtttgccgtgttcaactagtgcacagtggaactcgtattcgacaagcatttggaaaactgttgaaatcaattcctttagatgttgtcctaagcaataacaatcacacagaaattcaagaaatttctttagcattaagaagtcacatgagtaaagcaccaagtaatacattccacccccaagatttctctgatgttattagttttattttgtatgggaactctcatagaacagggaaggacaattggttggaaagactgttctatagctgccagagactggataagcgtgaccagtcaacaattccacgcaatctcctgaagacagatgctgtcctttggcagtgggccatatgggaagctgcacaattcactgttctttctaagctgagaaccccactgggcagagctcaagacaccttccagacaattgaaggtatcattcgaagtctcgcagctcacacattaaaccctgatcaggatgttagtcagtggacaactgcagacaatgatgaaggccatggtaacaaccaacttagacttgttcttcttctgcagtatctggaaaatctggagaaattaatgtataatgcatacgagggatgtgctaatgcattaacttcacctcccaaggtcattagaacttttttctataccaatcgccaaacttgtcaggactggctaacgcggattcgactctccatcatgagggtaggattgttggcaggccagcctgcagtgacagtgagacatggctttgacttgcttacagagatgaaaacaaccagcctatctcaggggaatgaattggaagtaaccattatgatggtggtagaagcattatgtgaacttcattgtcctgaagctatacagggaattgctgtctggtcatcatctattgttggaaaaaatcttctgtggattaactcagtggctcaacaggctgaagggaggtttgaaaaggcctctgtggagtaccaggaacacctgtgtgccatgacaggtgttgattgctgcatctccagctttgacaaatcggtgctcaccttagccaatgctgggcgtaacagtgccagcccgaaacattctctgaatggtgaatccagaaaaactgtgctgtccaaaccgactgactcttcccctgaggttataaattatttaggaaataaagcatgtgagtgctacatctcaattgccgattgggctgctgtgcaggaatggcagaacgctatccatgacttgaaaaagagtaccagtagcacttccctcaacctgaaagctgacttcaactatataaaatcattaagcagctttgagtctggaaaatttgttgaatgtaccgagcagttagaattgttaccaggagaaaatatcaatctacttgctggaggatcaaaagaaaaaatagacatgaaaaaactgcttcctaacatgttaagtccggatccgagggaacttcagaaatccattgaagttcaattgttaagaagttctgtttgtttggcaactgctttaaacccgatagaacaagatcagaagtggcagtctataactgaaaatgtggtaaagtacttgaagcaaacatcccgcatcgctattggacctctgagactttctactttaacagtttcacagtctttgccagttctaagtaccttgcagctgtattgctcatctgctttggagaacacagtttctaacagactttcaacagaggactgtcttattccactcttcagtgaagctttacgttcatgtaaacagcatgacgtgaggccatggatgcaggcattaaggtatactatgtaccagaatcagttgttggagaaaattaaagaacaaacagtcccaattagaagccatctcatggaattaggtctaacagcagcaaaatttgctagaaaacgagggaatgtgtcccttgcaacaagactgctggcacagtgcagtgaagttcagtaaaattccacacaacaactag

SEQ ID NO: 45 - DNA, 5022 bp, synthetic construct
  misc_feature 1..5022: note = 5002 nt DNA product
  source 1..5022: mol_type = other DNA
caataatacgactcactatagggagaaaaatcgagggtctcccctagttgttgtgtggaattatgtcttattctgatgagtctcgactgtcgaatcttcttcggaggatcacccgggaagacgacagagaccgaagattggctactgtaaagcagttgaaagaatttattcagcaaccagaaaataagctggtactagttaaacaattggataatatcttggctgctgtacatgacgtgcttaatgaaagtagcaaattgcttcaggagttgagacaggagggagcttgctgtcttggccttctttgtgcttctctgagctatgaggctgagaagatcttcaagtggatttttagcaaatttagctcatctgcaaaagatgaagttaaactcctctacttatgtgccacctacaaagcactagagactgtaggagaaaagaaagccttttcatctgtaatgcagcttgtaatgaccagcctgcagtctattcttgaaaatgtggatacaccagaattgctttgtaaatgtgttaagtgcattcttttggtggctcgatgttaccctcatattttcagcactaattttagggatacagttgatatattagttggatggcatatagatcatactcagaaaccttcgctcacgcagcaggtatctgggtggttgcagagtttggagccattttgggtagctgatcttgcattttctactactcttcttggtcagtttctggaagacatggaagcatatgctgaggacctcagccatgtggcctctggggaatcagtggatgaagatgtccctcctccatcagtgtcattaccaaagctggctgcacttctccgggtatttagtactgtggtgaggagcattggggaacgcttcagcccaattcggggtcctccaattactgaggcatatgtaacagatgttctgtacagagtaatgagatgtgtgacggctgcaaaccaggtgtttttttctgaggctgtgttgacagctgctaatgagtgtgttggtgttttgctcggcagcttggatcctagcatgactatacattgtgacatggtcattacatatggattagaccaactggagaattgccagacttgtggtaccgattatatcatctcagtcttgaatttactcacgctgattgttgaacagataaatacgaaactgccatcatcatttgtagaaaaactgtttataccatcatctaaactactattcttgcgttatcataaagaaaaagaggttgttgctgtagcccatgctgtttatcaagcagtgctcagcttgaagaatattcctgttttggagactgcctataagttaatattgggagaaatgacttgtgccctaaacaacctcctacacagtctacaacttcctgaggcctgttctgaaataaaacatgaggcttttaagaatcatgtgttcaatgtagacaatgcaaaatttgtagttatatttgacctcagtgccctgactacaattggaaatgccaaaaactcactaatagggatgtgggcgctatctccaactgtctttgcacttctgagtaagaatctgatgattgtgcacagtgacctggctgttcacttccctgccattcagtatgctgtgctctacacattgtattctcattgtaccaggcatgatcactttatctctagtagcctcagttcttcctctccttctttgtttgatggagctgtgattagcactgtaactacggctacaaagaaacatttctcaattatattaaatcttctgggaatattacttaagaaagataaccttaaccaggacacgaggaaactgttaatgacttgggctttggaagcagctgttttaatgaagaagtctgaaacatacgcacctttattctctcttccgtctttccataaattttgcaaaggccttttagccaacactctcgttgaagatgtgaatatctgtctgcaggcatgcagcagtctacatgctctgtcctcttccttgccagatgatcttttacagagatgtgtcgatgtttgccgtgttcaactagtgcacagtggaactcgtattcgacaagcatttggaaaactgttgaaatcaattcctttagatgttgtcctaagcaataacaatcacacagaaattcaagaaatttctttagcattaagaagtcacatgagtaaagcaccaagtaatacattccacccccaagatttctctgatgttattagttttattttgtatgggaactctcatagaacagggaaggacaattggttggaaagactgttctatagctgccagagactggataagcgtgaccagtcaacaattccacgcaatctcctgaagacagatgctgtcctttggcagtgggccatatgggaagctgcacaattcactgttctttctaagctgagaaccccactgggcagagctcaagacaccttccagacaattgaaggtatcattcgaagtctcgcagctcacacattaaaccctgatcaggatgttagtcagtggacaactgcagacaatgatgaaggccatggtaacaaccaacttagacttgttcttcttctgcagtatctggaaaatctggagaaattaatgtataatgcatacgagggatgtgctaatgcattaacttcacctcccaaggtcattagaacttttttctataccaatcgccaaacttgtcaggactggctaacgcggattcgactctccatcatgagggtaggattgttggcaggccagcctgcagtgacagtgagacatggctttgacttgcttacagagatgaaaacaaccagcctatctcaggggaatgaattggaagtaaccattatgatggtggtagaagcattatgtgaacttcattgtcctgaagctatacagggaattgctgtctggtcatcatctattgttggaaaaaatcttctgtggattaactcagtggctcaacaggctgaagggaggtttgaaaaggcctctgtggagtaccaggaacacctgtgtgccatgacaggtgttgattgctgcatctccagctttgacaaatcggtgctcaccttagccaatgctgggcgtaacagtgccagcccgaaacattctctgaatggtgaatccagaaaaactgtgctgtccaaaccgactgactcttcccctgaggttataaattatttaggaaataaagcatgtgagtgctacatctcaattgccgattgggctgctgtgcaggaatggcagaacgctatccatgacttgaaaaagagtaccagtagcacttccctcaacctgaaagctgacttcaactatataaaatcattaagcagctttgagtctggaaaatttgttgaatgtaccgagcagttagaattgttaccaggagaaaatatcaatctacttgctggaggatcaaaagaaaaaatagacatgaaaaaactgcttcctaacatgttaagtccggatccgagggaacttcagaaatccattgaagttcaattgttaagaagttctgtttgtttggcaactgctttaaacccgatagaacaagatcagaagtggcagtctataactgaaaatgtggtaaagtacttgaagcaaacatcccgcatcgctattggacctctgagactttctactttaacagtttcacagtctttgccagttctaagtaccttgcagctgtattgctcatctgctttggagaacacagtttctaacagactttcaacagaggactgtcttattccactcttcagtgaagctttacgttcatgtaaacagcatgacgtgaggccatggatgcaggcattaaggtatactatgtaccagaatcagttgttggagaaaattaaagaacaaacagtcccaattagaagccatctcatggaattaggtctaacagcagcaaaatttgctagaaaacgagggaatgtgtcccttgcaacaagactgctggcacagtgcagtgaagttcagctgggaaagaccaccactgcacaggatttagtccaacattttaaaaaactatcaacccaaggtcaagtggatgaaaaatgggggcccgaacttgatattgaaaaaaccaaattgctttatacagcaggccagtcaacacatgcaatggaaatgttgagttcttgtgccatatctttctgcaagtctgtgaaagctgaatatgcagttgctaaatcaattctgacactggctaaatggatccaggcagaatggaaagagatttcaggacagctgaaacaggtttacagagctcagcaccaacagaacttcacaggtctttctactttgtctaaaaacatactcactctaatagaactgccatctgttaatacgatggaagaagagtatcctcggatcgagagtgaatctacagtgcatattggagttggagaacctgacttcattttgggacagttgtatcacctgtcttcagtacaggcacctgaagtagccaaatcttgggcagcgttggccagctgggcttataggtggggcagaaaggtggttgacaatgccagtcagggagaaggtgttcgtctgctgcctagagaaaaatctgaagttcagaatctacttccagacactataactgaggaagagaaagagagaatatatggtattcttggacaggctgtgtgtcggccggcggggattcaggatgaagatataacacttcagataactgagagtgaagacaacgaagaagatgacatggttgatgttatctggcgtcagttgatatcaagctgcccatggctttcagaacttgatgaaagtgcaactgaaggagttattaaagtgtggaggaaagttgtagatagaatattcagcctgtacaaactctcttgcagtgcatactttactttccttaaactcaacgctggtcaaattcctttagatgaggatgaccctaggctgcatttaagtcacagagtggaacagagcactgatgacatgattgtgtaaaattccacacaacaactag